European Patent Application EP 4 772 640 A1, published July 8, 2026. Title: 一种微环DNA制备方法及其用途. Applicant: 星尘股份有限公司. The sequence listing filed with the application follows.

SEQUENCE LISTING (3 sequences)

SEQ ID NO: 1 - protein, 188 aa, synthetic construct
  source 1..188: note = CinH resolvase amino acid sequence
MKGQKVGYVRVSSVEQNTGRQLEGIEVDRIFVDRASGKNTDRPKFQEMLNYVREGDRVIVHSMDRFARSLKDLVTEVDKLVKRGIAIQFVKENITFTAQSTPMDNLMLQLMGAFAQFEREIILERQKEGIKIAAAQGKYKGRVHKLNPDQAKALLQAWKEGKYSSKVDLAKAFGISRQAVYRYLKQIN

SEQ ID NO: 2 - DNA, 567 bp, synthetic construct
  source 1..567: mol_type = other DNA; note = CinH resolvase nucleotide sequence
gtgaaaggccaaaaagtagggtatgtgcgagtgagttcggtcgagcaaaatacagggcgtcaacttgagggaattgaagtcgaccggatttttgttgaccgtgcttcgggtaaaaataccgaccgaccgaaatttcaagaaatgttgaactatgtccgggaaggggatagggtgattgtacattccatggatcgttttgcacgaagtctaaaagatttggtcactgaagtagataaactggtcaaaagagggatcgccatccagtttgtaaaagagaatattacttttactgcccaatccacgccgatggataatttgatgctgcaactgatgggtgcttttgctcaattcgagcgggaaattatcttagaacgtcagaaagaagggattaagatcgcagcagctcagggcaaatataaaggtcgtgtccataaattgaatccagatcaagctaaagcattactgcaagcctggaaagaagggaagtattcatcaaaagttgatctggcaaaagcgtttggtatcagtagacaggctgtctatcggtatttaaaacaaattaattag

SEQ ID NO: 3 - DNA, 119 bp, synthetic construct
  source 1..119: mol_type = other DNA; note = RS2 sequence
cgttactttggggtataccctaaagttacaatataaaagttcttaaaactatgtaacatttaaatgatttttaaccatatataacatgtaactttgatatttaaagtttataatttacg